European Patent Specification EP 3 389 699 B1, published May 1, 2024. Title: Chimeric and humanized anti-human CTLA4 monoclonal antibodies and uses thereof. Applicant: OncoImmune, Inc. Liu, Yang Zheng, Pan Devenport, Martin. The sequence listing filed with the application follows.

SEQUENCE LISTING (73 sequences)

SEQ ID NO: 1 - protein, 107 aa, Mus musculus
DIQMTQSPASLSVSVGETVTITCRASENIYSNLAWYQQKQGKSPQLLVYAATNLADGVPSRFSGSGSGTQYSLKINSLQSEDFGTYFCQHLWGTPYTFGGGTKLEIK

SEQ ID NO: 2 - protein, 125 aa, Mus musculus
QVQLKESGPGLVAPSQSLSITCTVSGFSLTSYGLSWVRQPPGKGLEWLGVIWYDGNTNFHSALISRLTISKDNSKSQVFLELNSLQTDDTATYYCAKTEGHYYGSNYGYYALDYWGQGTSVTVSS

SEQ ID NO: 3 - protein, 329 aa, Homo sapiens
ASTKGPSVFPLAPSSKSTSGGTAALGCLVKDYFPEPVTVSWNSGALTSGVHTFPAVLQSSGLYSLSSVVTVPSSSLGTQTYICNVNHKPSNTKVDKKVEPKSCDKTHTCPPCPAPELLGGPSVFLFPPKPKDTLMISRTPEVTCVVVDVSHEDPEVKFNWYVDGVEVHNAKTKPREEQYNSTYRVVSVLTVLHQDWLNGKEYKCKVSNKALPAPIEKTISKAKGQPREPQVYTLPPSRDELTKNQVSLTCLVKGFYPSDIAVEWESNGQPENNYKTTPPVLDSDGSFFLYSKLTVDKSRWQQGNVFSCSVMHEALHNHYTQKSLSLSPG

SEQ ID NO: 4 - protein, 329 aa, Artificial Sequence
  Engineered fragment
ASTKGPSVFPLAPSSKSTSGGTAALGCLVKDYFPEPVTVSWNSGALTSGVHTFPAVLQSSGLYSLSSVVTVPSSSLGTQTYICNVNHKPSNTKVDKKVEPKSCDKTHTCPPCPAPELLGGPSVFLFPPKPKDTLYITREPEVTCVVVDVSHEDPEVKFNWYVDGVEVHNAKTKPREEQYNATYRVVSVLTVLHQDWLNGKEYKCKVSNKALPAPIAATISKAKGQPREPQVYTLPPSRDELTKNQVSLTCLVKGFYPSDIAVEWESNGQPENNYKTTPPVLDSDGSFFLYSKLTVDKSRWQQGNVFSCSVMHEALHNHYTQKSLSLSPG

SEQ ID NO: 5 - DNA, 1437 bp, Artificial Sequence
  Optimized fragment
atggaccccaagggcagcctgagctggagaatcctgctgttcctgagcctggccttcgagctgagctacggccaggtgcagctgaaagagtctggccctggcctggtggccccttcccagtccctgtctatcacctgtaccgtgtccggcttctccctgacctcctacggcctgtcttgggtgcgacagcctcctggcaagggcctggaatggctgggagtgatttggtacgacggcaacaccaacttccactccgccctgatctcccggctgaccatctccaaggacaactccaagtcccaggtgttcctggaactgaactccctgcagaccgacgacaccgccacctactactgcgctaagaccgagggccactactacggctccaactacggctactacgccctggactattggggccagggcacctccgtgaccgtgtcctctgctagcaccaagggccccagcgtgttccctctggcccccagcagcaagagcaccagcggcggaaccgccgccctgggctgcctggtgaaggactacttccccgagcccgtgaccgtgtcctggaacagcggcgctctgaccagcggagtgcacaccttccctgccgtgctgcagagcagcggcctgtactccctgagcagcgtggtgaccgtgcccagcagcagcctgggcacccagacctacatctgcaacgtgaaccacaagccctccaacaccaaggtggacaagaaggtggagcctaagagctgcgacaagacccacacctgccctccctgccccgcccccgagctgctgggcggacccagcgtgttcctgttccctcccaagcccaaggacaccctgtacatcacccgcgaacccgaggtgacctgcgtggtggtggacgtgagccacgaggaccccgaggtgaagttcaactggtacgtggacggcgtggaggtgcacaacgccaagaccaagcctcgggaggagcagtacaacgccacctaccgcgtggtgagcgtgctgaccgtgctgcaccaggactggctgaacggcaaggagtacaagtgcaaggtgagcaacaaggccctgcccgctcccatcgcagccaccatcagcaaggccaagggccagccccgggagcctcaggtgtacaccctgccccccagccgcgacgagctgaccaagaaccaggtgagcctgacctgcctggtgaagggcttctacccctccgacatcgccgtggagtgggagagcaacggccagcctgagaacaactacaagaccacccctcccgtgctggacagcgacggcagcttcttcctgtacagcaagctgaccgtggacaagtcccggtggcagcagggcaacgtgttcagctgcagcgtgatgcacgaggccctgcacaaccactacacccagaagagcctgagcctgagccccggatag

SEQ ID NO: 6 - protein, 478 aa, Artificial Sequence
  Optimized fragment
MDPKGSLSWRILLFLSLAFELSYGQVQLKESGPGLVAPSQSLSITCTVSGFSLTSYGLSWVRQPPGKGLEWLGVIWYDGNTNFHSALISRLTISKDNSKSQVFLELNSLQTDDTATYYCAKTEGHYYGSNYGYYALDYWGQGTSVTVSSASTKGPSVFPLAPSSKSTSGGTAALGCLVKDYFPEPVTVSWNSGALTSGVHTFPAVLQSSGLYSLSSVVTVPSSSLGTQTYICNVNHKPSNTKVDKKVEPKSCDKTHTCPPCPAPELLGGPSVFLFPPKPKDTLYITREPEVTCVVVDVSHEDPEVKFNWYVDGVEVHNAKTKPREEQYNATYRVVSVLTVLHQDWLNGKEYKCKVSNKALPAPIAATISKAKGQPREPQVYTLPPSRDELTKNQVSLTCLVKGFYPSDIAVEWESNGQPENNYKTTPPVLDSDGSFFLYSKLTVDKSRWQQGNVFSCSVMHEALHNHYTQKSLSLSPG

SEQ ID NO: 7 - DNA, 705 bp, Artificial Sequence
  Optimized fragment
atggagaccgacaccctgctgctctgggtgctgctgctctgggtgcccggctccaccggagacatccagatgacccagtcccccgcctccctgtctgtgtctgtgggcgagacagtgaccatcacctgtcgggcctccgagaacatctactccaacctggcctggtatcagcagaagcagggcaagtcccctcagctgctggtgtacgccgccaccaatctggctgatggcgtgccctccagattctccggctctggctctggcacccagtactccctgaagatcaactccctgcagtccgaggacttcggcacctacttttgccagcacctgtggggcaccccctacacctttggcggcggaacaaagctggaaatcaagcggaccgtggccgcccccagcgtgttcatcttccctcccagcgacgagcagctgaagtctggcaccgccagcgtggtgtgcctgctgaacaacttctacccccgcgaggccaaggtgcagtggaaggtggacaacgccctgcagagcggcaacagccaggagagcgtgaccgagcaggactccaaggacagcacctacagcctgagcagcaccctgaccctgagcaaggccgactacgagaagcacaaggtgtacgcctgcgaggtgacccaccagggactgtctagccccgtgaccaagagcttcaaccggggcgagtgctaa

SEQ ID NO: 8 - protein, 234 aa, Artificial Sequence
  Chimeric
METDTLLLWVLLLWVPGSTGDIQMTQSPASLSVSVGETVTITCRASENIYSNLAWYQQKQGKSPQLLVYAATNLADGVPSRFSGSGSGTQYSLKINSLQSEDFGTYFCQHLWGTPYTFGGGTKLEIKRTVAAPSVFIFPPSDEQLKSGTASVVCLLNNFYPREAKVQWKVDNALQSGNSQESVTEQDSKDSTYSLSSTLTLSKADYEKHKVYACEVTHQGLSSPVTKSFNRGEC

SEQ ID NO: 9 - protein, 478 aa, Artificial Sequence
  Humanized antibody fragment
MDPKGSLSWRILLFLSLAFELSYGQVQLQESGPGLVKPSETLSLTCTVSGFSLTSYGLSWIRQPPGKGLEWIGYIWYDGNTNFHPSLKSRVTISKDTSKNQFSLKLSSVTAADTAVYYCAKTEGHYYGSNYGYYALDYWGQGTSVTVSSASTKGPSVFPLAPSSKSTSGGTAALGCLVKDYFPEPVTVSWNSGALTSGVHTFPAVLQSSGLYSLSSVVTVPSSSLGTQTYICNVNHKPSNTKVDKKVEPKSCDKTHTCPPCPAPELLGGPSVFLFPPKPKDTLYITREPEVTCVVVDVSHEDPEVKFNWYVDGVEVHNAKTKPREEQYNATYRVVSVLTVLHQDWLNGKEYKCKVSNKALPAPIAATISKAKGQPREPQVYTLPPSRDELTKNQVSLTCLVKGFYPSDIAVEWESNGQPENNYKTTPPVLDSDGSFFLYSKLTVDKSRWQQGNVFSCSVMHEALHNHYTQKSLSLSPG

SEQ ID NO: 10 - DNA, 1440 bp, Artificial Sequence
  Humanized antibody fragment
atggaccccaagggcagcctgagctggagaatcctgctgttcctgagcctggccttcgagctgagctacggccaggtgcagctgcaggaatctggccctggcctcgtgaagccctccgagacactgtctctgacctgcaccgtgtccggcttctccctgacctcctacggcctgtcttggatcagacagccccctggcaagggcctggaatggatcggctacatttggtacgacggcaacaccaacttccaccccagcctgaagtccagagtgaccatctccaaggacacctccaagaaccagttctctctgaagctgtcctccgtgaccgccgctgacaccgccgtgtactactgtgctaagaccgagggccactactacggctccaactacggctactacgccctggactattggggccagggcacctctgtgaccgtgtcctctgctagcaccaagggccccagcgtgttccctctggcccccagcagcaagagcaccagcggcggaaccgccgccctgggctgcctggtgaaggactacttccccgagcccgtgaccgtgtcctggaacagcggcgctctgaccagcggagtgcacaccttccctgccgtgctgcagagcagcggcctgtactccctgagcagcgtggtgaccgtgcccagcagcagcctgggcacccagacctacatctgcaacgtgaaccacaagccctccaacaccaaggtggacaagaaggtggagcctaagagctgcgacaagacccacacctgccctccctgccccgcccccgagctgctgggcggacccagcgtgttcctgttccctcccaagcccaaggacaccctgtacatcacccgcgaacccgaggtgacctgcgtggtggtggacgtgagccacgaggaccccgaggtgaagttcaactggtacgtggacggcgtggaggtgcacaacgccaagaccaagcctcgggaggagcagtacaacgccacctaccgcgtggtgagcgtgctgaccgtgctgcaccaggactggctgaacggcaaggagtacaagtgcaaggtgagcaacaaggccctgcccgctcccatcgcagccaccatcagcaaggccaagggccagccccgggagcctcaggtgtacaccctgccccccagccgcgacgagctgaccaagaaccaggtgagcctgacctgcctggtgaagggcttctacccctccgacatcgccgtggagtgggagagcaacggccagcctgagaacaactacaagaccacccctcccgtgctggacagcgacggcagcttcttcctgtacagcaagctgaccgtggacaagtcccggtggcagcagggcaacgtgttcagctgcagcgtgatgcacgaggccctgcacaaccactacacccagaagagcctgagcctgagccccggatagtaa

SEQ ID NO: 11 - protein, 478 aa, Artificial Sequence
  Humanized antibody fragment
MDPKGSLSWRILLFLSLAFELSYGQVQLQESGPGLVKPSETLSLTCTVSGFSLTSYGLSWIRQPPGKGLEWIGYIWYDGNTNFHSSLKSRVTISKDTSKSQVSLKLSSVTAADTAVYYCAKTEGHYYGSNYGYYALDYWGQGTLVTVSSASTKGPSVFPLAPSSKSTSGGTAALGCLVKDYFPEPVTVSWNSGALTSGVHTFPAVLQSSGLYSLSSVVTVPSSSLGTQTYICNVNHKPSNTKVDKKVEPKSCDKTHTCPPCPAPELLGGPSVFLFPPKPKDTLYITREPEVTCVVVDVSHEDPEVKFNWYVDGVEVHNAKTKPREEQYNATYRVVSVLTVLHQDWLNGKEYKCKVSNKALPAPIAATISKAKGQPREPQVYTLPPSRDELTKNQVSLTCLVKGFYPSDIAVEWESNGQPENNYKTTPPVLDSDGSFFLYSKLTVDKSRWQQGNVFSCSVMHEALHNHYTQKSLSLSPG

SEQ ID NO: 12 - DNA, 1440 bp, Artificial Sequence
  Humanized antibody
atggaccccaagggcagcctgagctggagaatcctgctgttcctgagcctggccttcgagctgagctacggccaggtgcagctgcaggaatctggccctggcctcgtgaagccctccgagacactgtctctgacctgcaccgtgtccggcttctccctgacctcctacggcctgtcttggatcagacagccccctggcaagggcctggaatggatcggctacatttggtacgacggcaacaccaacttccactcctccctgaagtccagagtgaccatctccaaggacacctccaagtcccaggtgtctctgaagctgtcctccgtgaccgccgctgacaccgccgtgtactactgtgctaagaccgagggccactactacggctccaactacggctactacgccctggactattggggccagggcaccctcgtgaccgtgtcctctgctagcaccaagggccccagcgtgttccctctggcccccagcagcaagagcaccagcggcggaaccgccgccctgggctgcctggtgaaggactacttccccgagcccgtgaccgtgtcctggaacagcggcgctctgaccagcggagtgcacaccttccctgccgtgctgcagagcagcggcctgtactccctgagcagcgtggtgaccgtgcccagcagcagcctgggcacccagacctacatctgcaacgtgaaccacaagccctccaacaccaaggtggacaagaaggtggagcctaagagctgcgacaagacccacacctgccctccctgccccgcccccgagctgctgggcggacccagcgtgttcctgttccctcccaagcccaaggacaccctgtacatcacccgcgaacccgaggtgacctgcgtggtggtggacgtgagccacgaggaccccgaggtgaagttcaactggtacgtggacggcgtggaggtgcacaacgccaagaccaagcctcgggaggagcagtacaacgccacctaccgcgtggtgagcgtgctgaccgtgctgcaccaggactggctgaacggcaaggagtacaagtgcaaggtgagcaacaaggccctgcccgctcccatcgcagccaccatcagcaaggccaagggccagccccgggagcctcaggtgtacaccctgccccccagccgcgacgagctgaccaagaaccaggtgagcctgacctgcctggtgaagggcttctacccctccgacatcgccgtggagtgggagagcaacggccagcctgagaacaactacaagaccacccctcccgtgctggacagcgacggcagcttcttcctgtacagcaagctgaccgtggacaagtcccggtggcagcagggcaacgtgttcagctgcagcgtgatgcacgaggccctgcacaaccactacacccagaagagcctgagcctgagccccggatagtaa

SEQ ID NO: 13 - protein, 478 aa, Artificial Sequence
  Humanized antibody
MDPKGSLSWRILLFLSLAFELSYGQVQLQESGPGLVKPSETLSLTCTVSGFSLTSYGLSWIRQPPGKGLEWIGYIWYDGNTNFHSPLKSRVTISVDTSKNQFSLKLSSVTAADTAVYYCAKTEGHYYGSNYGYYALDYWGQGTLVTVSSASTKGPSVFPLAPSSKSTSGGTAALGCLVKDYFPEPVTVSWNSGALTSGVHTFPAVLQSSGLYSLSSVVTVPSSSLGTQTYICNVNHKPSNTKVDKKVEPKSCDKTHTCPPCPAPELLGGPSVFLFPPKPKDTLYITREPEVTCVVVDVSHEDPEVKFNWYVDGVEVHNAKTKPREEQYNATYRVVSVLTVLHQDWLNGKEYKCKVSNKALPAPIAATISKAKGQPREPQVYTLPPSRDELTKNQVSLTCLVKGFYPSDIAVEWESNGQPENNYKTTPPVLDSDGSFFLYSKLTVDKSRWQQGNVFSCSVMHEALHNHYTQKSLSLSPG

SEQ ID NO: 14 - DNA, 1440 bp, Artificial Sequence
  Humanized antibody
atggaccccaagggcagcctgagctggagaatcctgctgttcctgagcctggccttcgagctgagctacggccaggtgcagctgcaggaatctggccctggcctcgtgaagccctccgagacactgtctctgacctgcaccgtgtccggcttctccctgacctcctacggcctgtcttggatcagacagccccctggcaagggcctggaatggatcggctacatttggtacgacggcaacaccaacttccactccccactgaagtccagagtgaccatctccgtggacacctccaagaaccagttctctctgaagctgtcctccgtgaccgccgctgacaccgccgtgtactactgtgctaagaccgagggccactactacggctccaactacggctactacgccctggactattggggccagggcaccctcgtgaccgtgtcctctgctagcaccaagggccccagcgtgttccctctggcccccagcagcaagagcaccagcggcggaaccgccgccctgggctgcctggtgaaggactacttccccgagcccgtgaccgtgtcctggaacagcggcgctctgaccagcggagtgcacaccttccctgccgtgctgcagagcagcggcctgtactccctgagcagcgtggtgaccgtgcccagcagcagcctgggcacccagacctacatctgcaacgtgaaccacaagccctccaacaccaaggtggacaagaaggtggagcctaagagctgcgacaagacccacacctgccctccctgccccgcccccgagctgctgggcggacccagcgtgttcctgttccctcccaagcccaaggacaccctgtacatcacccgcgaacccgaggtgacctgcgtggtggtggacgtgagccacgaggaccccgaggtgaagttcaactggtacgtggacggcgtggaggtgcacaacgccaagaccaagcctcgggaggagcagtacaacgccacctaccgcgtggtgagcgtgctgaccgtgctgcaccaggactggctgaacggcaaggagtacaagtgcaaggtgagcaacaaggccctgcccgctcccatcgcagccaccatcagcaaggccaagggccagccccgggagcctcaggtgtacaccctgccccccagccgcgacgagctgaccaagaaccaggtgagcctgacctgcctggtgaagggcttctacccctccgacatcgccgtggagtgggagagcaacggccagcctgagaacaactacaagaccacccctcccgtgctggacagcgacggcagcttcttcctgtacagcaagctgaccgtggacaagtcccggtggcagcagggcaacgtgttcagctgcagcgtgatgcacgaggccctgcacaaccactacacccagaagagcctgagcctgagccccggatagtaa

SEQ ID NO: 15 - protein, 234 aa, Artificial Sequence
  Humanized antibody
METDTLLLWVLLLWVPGSTGDIQMTQSPSSLSASVGDRVTITCRASENIYSNLAWYQQKPGKAPKLLLYAATNLQSGVPSRFSGSGSGTDFTLTISSLQPEDFATYYCQHLWGTPYTFGGGTKLEIKRTVAAPSVFIFPPSDEQLKSGTASVVCLLNNFYPREAKVQWKVDNALQSGNSQESVTEQDSKDSTYSLSSTLTLSKADYEKHKVYACEVTHQGLSSPVTKSFNRGEC

SEQ ID NO: 16 - DNA, 705 bp, Artificial Sequence
  Humanized antibody
atggagaccgacaccctgctgctctgggtgctgctgctctgggtgcccggctccaccggagacatccagatgacccagtccccctccagcctgtctgcctctgtgggcgacagagtgaccatcacctgtcgggcctccgagaacatctactccaacctggcctggtatcagcagaagcccggcaaggcccctaagctgctgctgtacgccgccaccaatctgcagtctggcgtgccctccagattctccggctctggctctggcaccgactttaccctgaccatcagctccctgcagcccgaggacttcgccacctactactgccagcatctgtggggcaccccctacacctttggcggaggcaccaagctggaaatcaagcggaccgtggccgcccccagcgtgttcatcttccctcccagcgacgagcagctgaagtctggcaccgccagcgtggtgtgcctgctgaacaacttctacccccgcgaggccaaggtgcagtggaaggtggacaacgccctgcagagcggcaacagccaggagagcgtgaccgagcaggactccaaggacagcacctacagcctgagcagcaccctgaccctgagcaaggccgactacgagaagcacaaggtgtacgcctgcgaggtgacccaccagggactgtctagccccgtgaccaagagcttcaaccggggcgagtgctaa

SEQ ID NO: 17 - protein, 234 aa, Artificial Sequence
  Humanized Antibody
METDTLLLWVLLLWVPGSTGDIQMTQSPSSLSASVGDRVTITCRASENIYSNLAWYQQKQGKAPKLLLYAATNLQDGVPSRFSGSGSGTDYTLTISSLQPEDFATYFCQHLWGTPYTFGQGTKLEIKRTVAAPSVFIFPPSDEQLKSGTASVVCLLNNFYPREAKVQWKVDNALQSGNSQESVTEQDSKDSTYSLSSTLTLSKADYEKHKVYACEVTHQGLSSPVTKSFNRGEC

SEQ ID NO: 18 - DNA, 705 bp, Artificial Sequence
  Humanized antibody
atggagaccgacaccctgctgctctgggtgctgctgctctgggtgcccggctccaccggagacatccagatgacccagtccccctccagcctgtctgcctctgtgggcgacagagtgaccatcacctgtcgggcctccgagaacatctactccaacctggcctggtatcagcagaagcagggcaaggcccctaagctgctgctgtacgccgccaccaatctgcaggatggcgtgccctccagattctccggctctggctctggcaccgactacaccctgaccatcagctccctgcagcccgaggacttcgccacctacttttgccagcatctgtggggcaccccctacacctttggccagggcaccaagctggaaatcaagcggaccgtggccgcccccagcgtgttcatcttccctcccagcgacgagcagctgaagtctggcaccgccagcgtggtgtgcctgctgaacaacttctacccccgcgaggccaaggtgcagtggaaggtggacaacgccctgcagagcggcaacagccaggagagcgtgaccgagcaggactccaaggacagcacctacagcctgagcagcaccctgaccctgagcaaggccgactacgagaagcacaaggtgtacgcctgcgaggtgacccaccagggactgtctagccccgtgaccaagagcttcaaccggggcgagtgctaa

SEQ ID NO: 19 - protein, 234 aa, Artificial Sequence
  Humanized antibody
METDTLLLWVLLLWVPGSTGDIQMTQSPSSLSASVGDRVTITCRASENIYSNLAWYQQKPGKAPKLLIYAATSLQSGVPSRFSGSGSGTDFTLTISSLQPEDFATYYCQHLWGTPYTFGGGTKVEIKRTVAAPSVFIFPPSDEQLKSGTASVVCLLNNFYPREAKVQWKVDNALQSGNSQESVTEQDSKDSTYSLSSTLTLSKADYEKHKVYACEVTHQGLSSPVTKSFNRGEC

SEQ ID NO: 20 - DNA, 705 bp, Artificial Sequence
  Humanized antibody
atggagaccgacaccctgctgctctgggtgctgctgctctgggtgcccggctccaccggagacatccagatgacccagtccccctccagcctgtctgcctctgtgggcgacagagtgaccatcacctgtcgggcctccgagaacatctactccaacctggcctggtatcagcagaagcccggcaaggcccctaagctgctgatctacgccgccaccagtctgcagtctggcgtgccctccagattctccggctctggctctggcaccgactttaccctgaccatcagctccctgcagcccgaggacttcgccacctactactgccagcatctgtggggcaccccctacacctttggcggaggcaccaaggtggaaatcaagcggaccgtggccgcccccagcgtgttcatcttccctcccagcgacgagcagctgaagtctggcaccgccagcgtggtgtgcctgctgaacaacttctacccccgcgaggccaaggtgcagtggaaggtggacaacgccctgcagagcggcaacagccaggagagcgtgaccgagcaggactccaaggacagcacctacagcctgagcagcaccctgaccctgagcaaggccgactacgagaagcacaaggtgtacgcctgcgaggtgacccaccagggactgtctagccccgtgaccaagagcttcaaccggggcgagtgctaa

SEQ ID NO: 21 - protein, 11 aa, Artificial Sequence
  Peptide fragment
RASENIYSNLA

SEQ ID NO: 22 - protein, 7 aa, Artificial Sequence
  Peptide fragment
AATNLAD

SEQ ID NO: 23 - protein, 9 aa, Artificial Sequence
  Peptide fragment
QHLWGTPYT

SEQ ID NO: 24 - protein, 10 aa, Artificial Sequence
  Peptide fragment
GFSLTSYGLS

SEQ ID NO: 25 - protein, 17 aa, Artificial Sequence
  Peptide fragment
VIWYDGNTNFHSALISR

SEQ ID NO: 26 - protein, 17 aa, Artificial Sequence
  Peptide fragment
TEGHYYGSNYGYYALDY

SEQ ID NO: 27 - protein, 149 aa, Artificial Sequence
  Humanized antibody
MDPKGSLSWRILLFLSLAFELSYGQVQLQESGPGLVKPSETLSLTCTVSGFSLTSYGLSWIRQPPGKGLEWIGYIWYDGNTNFHPSLKSRVTISKDTSKNQFSLKLSSVTAADTAVYYCAKTEGHYYGSNYGYYALDYWGQGTSVTVSS

SEQ ID NO: 28 - protein, 149 aa, Artificial Sequence
  Humanized antibody
MDPKGSLSWRILLFLSLAFELSYGQVQLQESGPGLVKPSETLSLTCTVSGFSLTSYGLSWIRQPPGKGLEWIGYIWYDGNTNFHSSLKSRVTISKDTSKSQVSLKLSSVTAADTAVYYCAKTEGHYYGSNYGYYALDYWGQGTLVTVSS

SEQ ID NO: 29 - protein, 149 aa, Artificial Sequence
  Humanized antibody
MDPKGSLSWRILLFLSLAFELSYGQVQLQESGPGLVKPSETLSLTCTVSGFSLTSYGLSWIRQPPGKGLEWIGYIWYDGNTNFHSPLKSRVTISVDTSKNQFSLKLSSVTAADTAVYYCAKTEGHYYGSNYGYYALDYWGQGTLVTVSS

SEQ ID NO: 30 - protein, 127 aa, Artificial Sequence
  Humanized antibody
METDTLLLWVLLLWVPGSTGDIQMTQSPSSLSASVGDRVTITCRASENIYSNLAWYQQKPGKAPKLLLYAATNLQSGVPSRFSGSGSGTDFTLTISSLQPEDFATYYCQHLWGTPYTFGGGTKLEIK

SEQ ID NO: 31 - protein, 127 aa, Artificial Sequence
  Humanized antibody
METDTLLLWVLLLWVPGSTGDIQMTQSPSSLSASVGDRVTITCRASENIYSNLAWYQQKQGKAPKLLLYAATNLQDGVPSRFSGSGSGTDYTLTISSLQPEDFATYFCQHLWGTPYTFGQGTKLEIK

SEQ ID NO: 32 - protein, 127 aa, Artificial Sequence
  Humanized antibody
METDTLLLWVLLLWVPGSTGDIQMTQSPSSLSASVGDRVTITCRASENIYSNLAWYQQKPGKAPKLLIYAATSLQSGVPSRFSGSGSGTDFTLTISSLQPEDFATYYCQHLWGTPYTFGGGTKVEIK

SEQ ID NO: 33 - protein, 17 aa, Artificial Sequence
  Peptide fragment
YIWYDGNTNFHPSLKSR

SEQ ID NO: 34 - protein, 17 aa, Artificial Sequence
  Peptide fragment
YIWYDGNTNFHSSLKSR

SEQ ID NO: 35 - protein, 17 aa, Artificial Sequence
  Peptide fragment
YIWYDGNTNFHSPLKSR

SEQ ID NO: 36 - protein, 7 aa, Artificial Sequence
  Peptide fragment
AATNLQS

SEQ ID NO: 37 - protein, 7 aa, Artificial Sequence
  Peptide
AATNLQD

SEQ ID NO: 38 - protein, 7 aa, Artificial Sequence
  Peptide
AATSLQS

SEQ ID NO: 39 - protein, 358 aa, Artificial Sequence
  Fusion protein
AMHVAQPAVVLASSRGIASFVCEYASPGKATEVRVTVLRQADSQVTEVCAATYMMGNELTFLDDSICTGTSSGNQVNLTIQGLRAMDTGLYICKVELMYPPPYYLGIGNGTQIYVIDPEPCPDSDQEPKSSDKTHTSPPSPAPELLGGSSVFLFPPKPKDTLMISRTPEVTCVVVDVSHEDPEVKFNWYVDGVEVHNAKTKPREEQYNSTYRVVSVLTVLHQDWLNGKEYKCKVSNKALPAPIEKTISKAKGQPREPQVYTLPPSRDELTKNQVSLTCLVKGFYPSDIAVEWESNGQPENNYKTTPPVLDSDGSFFLYSKLTVDKSRWQQGNVFSCSVMHEALHNHYTQKSLSLSPGK

SEQ ID NO: 40 - protein, 357 aa, Artificial Sequence
  Fusion protein
IQVTQPSVVLASSRGIASFVCEYASPGKATEVRVTVLRQADSQVTEVCAATYMMGNELTFLDDSICTGTSSGNQVNLTIQGLRAMDTGLYICKVELMYPPPYYLGIGNGTQIYVIDPEPCPDSDQEPKSSDKTHTSPPSPAPELLGGSSVFLFPPKPKDTLMISRTPEVTCVVVDVSHEDPEVKFNWYVDGVEVHNAKTKPREEQYNSTYRVVSVLTVLHQDWLNGKEYKCKVSNKALPAPIEKTISKAKGQPREPQVYTLPPSRDELTKNQVSLTCLVKGFYPSDIAVEWESNGQPENNYKTTPPVLDSDGSFFLYSKLTVDKSRWQQGNVFSCSVMHEALHNHYTQKSLSLSPGK

SEQ ID NO: 41 - protein, 358 aa, Artificial Sequence
  Fusion protein
AMHVAQPAVVLASSHGLASFPCEYASPGKATEVRVTVLRQADSQVTEVCAATYMMGNELTFLDDSICTGTSSGNQVNLTIQGLRAMDTGLYICKVELMYPPPYYLGIGNGTQIYVIDPEPCPDSDQEPKSSDKTHTSPPSPAPELLGGSSVFLFPPKPKDTLMISRTPEVTCVVVDVSHEDPEVKFNWYVDGVEVHNAKTKPREEQYNSTYRVVSVLTVLHQDWLNGKEYKCKVSNKALPAPIEKTISKAKGQPREPQVYTLPPSRDELTKNQVSLTCLVKGFYPSDIAVEWESNGQPENNYKTTPPVLDSDGSFFLYSKLTVDKSRWQQGNVFSCSVMHEALHNHYTQKSLSLSPGK

SEQ ID NO: 42 - protein, 359 aa, Artificial Sequence
  Fusion protein
AMHVAQPAVVLASSRGIASFVCEYASPSHNTDEVRVTVLRQADSQVTEVCAATYMMGNELTFLDDSICTGTSSGNQVNLTIQGLRAMDTGLYICKVELMYPPPYYLGIGNGTQIYVIDPEPCPDSDQEPKSSDKTHTSPPSPAPELLGGSSVFLFPPKPKDTLMISRTPEVTCVVVDVSHEDPEVKFNWYVDGVEVHNAKTKPREEQYNSTYRVVSVLTVLHQDWLNGKEYKCKVSNKALPAPIEKTISKAKGQPREPQVYTLPPSRDELTKNQVSLTCLVKGFYPSDIAVEWESNGQPENNYKTTPPVLDSDGSFFLYSKLTVDKSRWQQGNVFSCSVMHEALHNHYTQKSLSLSPGK

SEQ ID NO: 43 - protein, 358 aa, Artificial Sequence
  Fusion protein
AMHVAQPAVVLASSRGIASFVCEYASPGKATEVRVTVLRTNDQMVTEVCAATYMMGNELTFLDDSICTGTSSGNQVNLTIQGLRAMDTGLYICKVELMYPPPYYLGIGNGTQIYVIDPEPCPDSDQEPKSSDKTHTSPPSPAPELLGGSSVFLFPPKPKDTLMISRTPEVTCVVVDVSHEDPEVKFNWYVDGVEVHNAKTKPREEQYNSTYRVVSVLTVLHQDWLNGKEYKCKVSNKALPAPIEKTISKAKGQPREPQVYTLPPSRDELTKNQVSLTCLVKGFYPSDIAVEWESNGQPENNYKTTPPVLDSDGSFFLYSKLTVDKSRWQQGNVFSCSVMHEALHNHYTQKSLSLSPGK

SEQ ID NO: 44 - protein, 358 aa, Artificial Sequence
  Fusion protein
AMHVAQPAVVLASSRGIASFVCEYASPGKATEVRVTVLRQADSQVTEVCAATFTEKNTVGFLDDSICTGTSSGNQVNLTIQGLRAMDTGLYICKVELMYPPPYYLGIGNGTQIYVIDPEPCPDSDQEPKSSDKTHTSPPSPAPELLGGSSVFLFPPKPKDTLMISRTPEVTCVVVDVSHEDPEVKFNWYVDGVEVHNAKTKPREEQYNSTYRVVSVLTVLHQDWLNGKEYKCKVSNKALPAPIEKTISKAKGQPREPQVYTLPPSRDELTKNQVSLTCLVKGFYPSDIAVEWESNGQPENNYKTTPPVLDSDGSFFLYSKLTVDKSRWQQGNVFSCSVMHEALHNHYTQKSLSLSPGK

SEQ ID NO: 45 - protein, 358 aa, Artificial Sequence
  Fusion protein
AMHVAQPAVVLASSRGIASFVCEYASPGKATEVRVTVLRQADSQVTEVCATTYMMGNELTFLDDSICTGTSSGNQVNLTIQGLRAMDTGLYICKVELMYPPPYYLGIGNGTQIYVIDPEPCPDSDQEPKSSDKTHTSPPSPAPELLGGSSVFLFPPKPKDTLMISRTPEVTCVVVDVSHEDPEVKFNWYVDGVEVHNAKTKPREEQYNSTYRVVSVLTVLHQDWLNGKEYKCKVSNKALPAPIEKTISKAKGQPREPQVYTLPPSRDELTKNQVSLTCLVKGFYPSDIAVEWESNGQPENNYKTTPPVLDSDGSFFLYSKLTVDKSRWQQGNVFSCSVMHEALHNHYTQKSLSLSPGK

SEQ ID NO: 46 - protein, 358 aa, Artificial Sequence
  Fusion protein
AMHVAQPAVVLASSRGIASFVCEYASPGKATEVRVTVLRQADSQVTEVCAATYMMGNELTFLDYPFCSGTSSGNQVNLTIQGLRAMDTGLYICKVELMYPPPYYLGIGNGTQIYVIDPEPCPDSDQEPKSSDKTHTSPPSPAPELLGGSSVFLFPPKPKDTLMISRTPEVTCVVVDVSHEDPEVKFNWYVDGVEVHNAKTKPREEQYNSTYRVVSVLTVLHQDWLNGKEYKCKVSNKALPAPIEKTISKAKGQPREPQVYTLPPSRDELTKNQVSLTCLVKGFYPSDIAVEWESNGQPENNYKTTPPVLDSDGSFFLYSKLTVDKSRWQQGNVFSCSVMHEALHNHYTQKSLSLSPGK

SEQ ID NO: 47 - protein, 358 aa, Artificial Sequence
  Fusion protein
AMHVAQPAVVLASSRGIASFVCEYASPGKATEVRVTVLRQADSQVTEVCAATYMMGNELTFLDDSICTGTFNESRVNLTIQGLRAMDTGLYICKVELMYPPPYYLGIGNGTQIYVIDPEPCPDSDQEPKSSDKTHTSPPSPAPELLGGSSVFLFPPKPKDTLMISRTPEVTCVVVDVSHEDPEVKFNWYVDGVEVHNAKTKPREEQYNSTYRVVSVLTVLHQDWLNGKEYKCKVSNKALPAPIEKTISKAKGQPREPQVYTLPPSRDELTKNQVSLTCLVKGFYPSDIAVEWESNGQPENNYKTTPPVLDSDGSFFLYSKLTVDKSRWQQGNVFSCSVMHEALHNHYTQKSLSLSPGK

SEQ ID NO: 48 - protein, 359 aa, Artificial Sequence
  Fusion protein
AMHVAQPAVVLASSRGIASFVCEYASPGKATEVRVTVLRQADSQVTEVCAATYMMGNELTFLDDSICTGTSSGNQVNLTIQGLRAMVDTGLYICKVELMYPPPYYLGIGNGTQIYVIDPEPCPDSDQEPKSSDKTHTSPPSPAPELLGGSSVFLFPPKPKDTLMISRTPEVTCVVVDVSHEDPEVKFNWYVDGVEVHNAKTKPREEQYNSTYRVVSVLTVLHQDWLNGKEYKCKVSNKALPAPIEKTISKAKGQPREPQVYTLPPSRDELTKNQVSLTCLVKGFYPSDIAVEWESNGQPENNYKTTPPVLDSDGSFFLYSKLTVDKSRWQQGNVFSCSVMHEALHNHYTQKSLSLSPGK

SEQ ID NO: 49 - protein, 359 aa, Artificial Sequence
  Fusion protein
AMHVAQPAVVLASSRGIASFVCEYASPGKATEVRVTVLRQADSQVTEVCAATYMMGNELTFLDDSICTGTSSGNQVNLTIQGLRAMMDTGLYLCKVELMYPPPYYLGIGNGTQIYVIDPEPCPDSDQEPKSSDKTHTSPPSPAPELLGGSSVFLFPPKPKDTLMISRTPEVTCVVVDVSHEDPEVKFNWYVDGVEVHNAKTKPREEQYNSTYRVVSVLTVLHQDWLNGKEYKCKVSNKALPAPIEKTISKAKGQPREPQVYTLPPSRDELTKNQVSLTCLVKGFYPSDIAVEWESNGQPENNYKTTPPVLDSDGSFFLYSKLTVDKSRWQQGNVFSCSVMHEALHNHYTQKSLSLSPGK

SEQ ID NO: 50 - protein, 358 aa, Artificial Sequence
  Fusion protein
AMHVAQPAVVLASSRGIASFVCEYASPGKATEVRVTVLRQADSQVTEVCAATYMMGNELTFLDDSICTGTSSGNQVNLTIQGLRAMDTGLYICKVELMYPPPYFVGMGNGTQIYVIDPEPCPDSDQEPKSSDKTHTSPPSPAPELLGGSSVFLFPPKPKDTLMISRTPEVTCVVVDVSHEDPEVKFNWYVDGVEVHNAKTKPREEQYNSTYRVVSVLTVLHQDWLNGKEYKCKVSNKALPAPIEKTISKAKGQPREPQVYTLPPSRDELTKNQVSLTCLVKGFYPSDIAVEWESNGQPENNYKTTPPVLDSDGSFFLYSKLTVDKSRWQQGNVFSCSVMHEALHNHYTQKSLSLSPGK

SEQ ID NO: 51 - protein, 357 aa, Artificial Sequence
  Fusion protein
IQVTQPSVVLASSRGIASFVCEYASPGKATEVRVTVLRQADSQVTEVCAATFTEKNTVGFLDDSICTGTFNESRVNLTIQGLRAMDTGLYICKVELMYPPPYFVGMGNGTQIYVIDPEPCPDSDQEPKSSDKTHTSPPSPAPELLGGSSVFLFPPKPKDTLMISRTPEVTCVVVDVSHEDPEVKFNWYVDGVEVHNAKTKPREEQYNSTYRVVSVLTVLHQDWLNGKEYKCKVSNKALPAPIEKTISKAKGQPREPQVYTLPPSRDELTKNQVSLTCLVKGFYPSDIAVEWESNGQPENNYKTTPPVLDSDGSFFLYSKLTVDKSRWQQGNVFSCSVMHEALHNHYTQKSLSLSPGK

SEQ ID NO: 52 - protein, 357 aa, Artificial Sequence
  Fusion protein
MHVAQPAVVLASSRGIASFVCEYASPGKYTEVRVTVLRQADSQVTEVCAATYMMGNELTFLDDSICTGTSSGNQVNLTIQGLRAMDTGLYICKVELMYPPPYFVGMGNGTQIYVIDPEPCPDSDQEPKSSDKTHTSPPSPAPELLGGSSVFLFPPKPKDTLMISRTPEVTCVVVDVSHEDPEVKFNWYVDGVEVHNAKTKPREEQYNSTYRVVSVLTVLHQDWLNGKEYKCKVSNKALPAPIEKTISKAKGQPREPQVYTLPPSRDELTKNQVSLTCLVKGFYPSDIAVEWESNGQPENNYKTTPPVLDSDGSFFLYSKLTVDKSRWQQGNVFSCSVMHEALHNHYTQKSLSLSPGK

SEQ ID NO: 53 - protein, 357 aa, Artificial Sequence
  Fusion protein
IQVTQPSVVLASSRGIASFVCEYASPGKATEVRVTVLRQADSQVTEVCAATFTEKNTVGFLDDSICTGTSSGNQVNLTIQGLRAMDTGLYICKVELMYPPPYFVGMGNGTQIYVIDPEPCPDSDQEPKSSDKTHTSPPSPAPELLGGSSVFLFPPKPKDTLMISRTPEVTCVVVDVSHEDPEVKFNWYVDGVEVHNAKTKPREEQYNSTYRVVSVLTVLHQDWLNGKEYKCKVSNKALPAPIEKTISKAKGQPREPQVYTLPPSRDELTKNQVSLTCLVKGFYPSDIAVEWESNGQPENNYKTTPPVLDSDGSFFLYSKLTVDKSRWQQGNVFSCSVMHEALHNHYTQKSLSLSPGK

SEQ ID NO: 54 - protein, 357 aa, Artificial Sequence
  Fusion protein
MHVAQPAVVLASSRGIASFVCEYASPGKYTEVRVTVLRQADSQVTEVCAATYMMGNELTFLDDSICTGTSSGNQVNLTIQGLRAMDTGLYICKVELMYPPPYYEGIGNGTQIYVIDPEPCPDSDQEPKSSDKTHTSPPSPAPELLGGSSVFLFPPKPKDTLMISRTPEVTCVVVDVSHEDPEVKFNWYVDGVEVHNAKTKPREEQYNSTYRVVSVLTVLHQDWLNGKEYKCKVSNKALPAPIEKTISKAKGQPREPQVYTLPPSRDELTKNQVSLTCLVKGFYPSDIAVEWESNGQPENNYKTTPPVLDSDGSFFLYSKLTVDKSRWQQGNVFSCSVMHEALHNHYTQKSLSLSPGK

SEQ ID NO: 55 - protein, 357 aa, Artificial Sequence
  Fusion protein
IQVTQPSVVLASSRGIASFVCEYASPGKATEVRVTVLRQADSQVTEVCAATFTEKNTVGFLDDSICTGTFNESRVNLTIQGLRAMDTGLYICKVELMYPPPYFVGMGNGTQIYVIDPEPCPDSDQEPKSSDKTHTSPPSPAPELLGGSSVFLFPPKPKDTLYITREPEVTCVVVDVSHEDPEVKFNWYVDGVEVHNAKTKPREEQYNSTYRVVSVLTVLHQDWLNGKEYKCKVSNKALPAPIEKTISKAKGQPREPQVYTLPPSRDELTKNQVSLTCLVKGFYPSDIAVEWESNGQPENNYKTTPPVLDSDGSFFLYSKLTVDKSRWQQGNVFSCSVMHEALHNHYTQKSLSLSPGK

SEQ ID NO: 56 - protein, 357 aa, Artificial Sequence
  Fusion protein
MHVAQPAVVLASSRGIASFVCEYASPGKYTEVRVTVLRQADSQVTEVCAATYMMGNELTFLDDSICTGTSSGNQVNLTIQGLRAMDTGLYICKVELMYPPPYFEGMGNGTQIYVIDPEPCPDSDQEPKSSDKTHTSPPSPAPELLGGSSVFLFPPKPKDTLMISRTPEVTCVVVDVSHEDPEVKFNWYVDGVEVHNAKTKPREEQYNSTYRVVSVLTVLHQDWLNGKEYKCKVSNKALPAPIEKTISKAKGQPREPQVYTLPPSRDELTKNQVSLTCLVKGFYPSDIAVEWESNGQPENNYKTTPPVLDSDGSFFLYSKLTVDKSRWQQGNVFSCSVMHEALHNHYTQKSLSLSPGK

SEQ ID NO: 57 - protein, 125 aa, Mus musculus; identical to SEQ ID NO: 2

SEQ ID NO: 58 - protein, 25 aa, Mus musculus
QVQLQESGPGLVKPSETLSLTCTVS

SEQ ID NO: 59 - protein, 14 aa, Mus musculus
WIRQPPGKGLEWIG

SEQ ID NO: 60 - protein, 31 aa, Mus musculus
VTISVDTSKNQFSLKLSSVTAADTAVYYCAR

SEQ ID NO: 61 - protein, 11 aa, Mus musculus
WGQGTLVTVSS

SEQ ID NO: 62 - protein, 125 aa, Artificial Sequence
  Humanized
QVQLQESGPGLVKPSETLSLTCTVSGFSLTSYGLSWIRQPPGKGLEWIGYIWYDGNTNFHPSLKSRVTISKDTSKNQFSLKLSSVTAADTAVYYCAKTEGHYYGSNYGYYALDYWGQGTSVTVSS

SEQ ID NO: 63 - protein, 125 aa, Artificial Sequence
  Humanized
QVQLQESGPGLVKPSETLSLTCTVSGFSLTSYGLSWIRQPPGKGLEWIGYIWYDGNTNFHSSLKSRVTISKDTSKSQVSLKLSSVTAADTAVYYCAKTEGHYYGSNYGYYALDYWGQGTLVTVSS

SEQ ID NO: 64 - protein, 125 aa, Artificial Sequence
  Humanized
QVQLQESGPGLVKPSETLSLTCTVSGFSLTSYGLSWIRQPPGKGLEWIGYIWYDGNTNFHSPLKSRVTISVDTSKNQFSLKLSSVTAADTAVYYCAKTEGHYYGSNYGYYALDYWGQGTLVTVSS

SEQ ID NO: 65 - protein, 107 aa, Mus musculus; identical to SEQ ID NO: 1

SEQ ID NO: 66 - protein, 23 aa, Mus musculus
DIQMTQSPSSLSASVGDRVTITC

SEQ ID NO: 67 - protein, 15 aa, Mus musculus
WYQQKPGKAPKLLIY

SEQ ID NO: 68 - protein, 32 aa, Mus musculus
GVPSRFSGSGSGTDFTLTISSLQPEDFATYYC

SEQ ID NO: 69 - protein, 10 aa, Mus musculus
FGQGTKLEIK

SEQ ID NO: 70 - protein, 107 aa, Artificial Sequence
  Humanized
DIQMTQSPSSLSASVGDRVTITCRASENIYSNLAWYQQKPGKAPKLLLYAATNLQSGVPSRFSGSGSGTDFTLTISSLQPEDFATYYCQHLWGTPYTFGGGTKLEIK

SEQ ID NO: 71 - protein, 107 aa, Artificial Sequence
  Humanized
DIQMTQSPSSLSASVGDRVTITCRASENIYSNLAWYQQKQGKAPKLLLYAATNLQDGVPSRFSGSGSGTDYTLTISSLQPEDFATYFCQHLWGTPYTFGQGTKLEIK

SEQ ID NO: 72 - protein, 107 aa, Artificial Sequence
  Humanized
DIQMTQSPSSLSASVGDRVTITCRASENIYSNLAWYQQKPGKAPKLLIYAATSLQSGVPSRFSGSGSGTDFTLTISSLQPEDFATYYCQHLWGTPYTFGGGTKVEIK

SEQ ID NO: 73 - protein, 124 aa, Homo sapiens [sequence omitted]